European Patent Application EP 4 353 742 A1, published April 17, 2024. Title: DEVELOPMENT OF NOVEL FGF21 VARIANTS, PRODUCTION TECHNIQUES AND USES THEREOF. Applicant: DOORCO KOREA CO.,LTD. The sequence listing filed with the application follows.

SEQUENCE LISTING (6 sequences)

SEQ ID NO: 1 - protein, 209 aa, FGF21_WT
MDSDETGFEHSGLWVSVLAGLLLGACQAHPIPDSSPLLQFGGQVRQRYLYTDDAQQTEAHLEIREDGTVGGAADQSPESLLQLKALKPGVIQILGVKTSRFLCQRPDGALYGSLHFDPEACSFRELLLEDGYNVYQSEAHGLPLHLPGNKSPHRDPAPRGPARFLPLPGLPPALPEPPGILAPQPPDVGSSDPLSMVGPSQGRSPSYAS

SEQ ID NO: 2 - protein, 181 aa, Artificial Sequence
  FGF21_mature
HPIPDSSPLLQFGGQVRQRYLYTDDAQQTEAHLEIREDGTVGGAADQSPESLLQLKALKPGVIQILGVKTSRFLCQRPDGALYGSLHFDPEACSFRELLLEDGYNVYQSEAHGLPLHLPGNKSPHRDPAPRGPARFLPLPGLPPALPEPPGILAPQPPDVGSSDPLSMVGPSQGRSPSYAS

SEQ ID NO: 3 - protein, 177 aa, Artificial Sequence
  FGF21_mature_N4
DSSPLLQFGGQVRQRYLYTDDAQQTEAHLEIREDGTVGGAADQSPESLLQLKALKPGVIQILGVKTSRFLCQRPDGALYGSLHFDPEACSFRELLLEDGYNVYQSEAHGLPLHLPGNKSPHRDPAPRGPARFLPLPGLPPALPEPPGILAPQPPDVGSSDPLSMVGPSQGRSPSYAS

SEQ ID NO: 4 - protein, 177 aa, Artificial Sequence
  FGF21_mature_N4_Q184E&Q201H&A208T
DSSPLLQFGGQVRQRYLYTDDAQQTEAHLEIREDGTVGGAADQSPESLLQLKALKPGVIQILGVKTSRFLCQRPDGALYGSLHFDPEACSFRELLLEDGYNVYQSEAHGLPLHLPGNKSPHRDPAPRGPARFLPLPGLPPALPEPPGILAPEPPDVGSSDPLSMVGPSHGRSPSYTS

SEQ ID NO: 5 - protein, 177 aa, Artificial Sequence
  FGF21_mature_N4_S195G&P199G&S200G
DSSPLLQFGGQVRQRYLYTDDAQQTEAHLEIREDGTVGGAADQSPESLLQLKALKPGVIQILGVKTSRFLCQRPDGALYGSLHFDPEACSFRELLLEDGYNVYQSEAHGLPLHLPGNKSPHRDPAPRGPARFLPLPGLPPALPEPPGILAPQPPDVGSSDPLGMVGGGQGRSPSYAS

SEQ ID NO: 6 - protein, 177 aa, Artificial Sequence
  FGF21_mature_N4_S195G&P199G&S200G&Q201H&A208T
DSSPLLQFGGQVRQRYLYTDDAQQTEAHLEIREDGTVGGAADQSPESLLQLKALKPGVIQILGVKTSRFLCQRPDGALYGSLHFDPEACSFRELLLEDGYNVYQSEAHGLPLHLPGNKSPHRDPAPRGPARFLPLPGLPPALPEPPGILAPQPPDVGSSDPLGMVGGGHGRSPSYTS